European Patent Specification EP 3 514 235 B1, published January 3, 2024. Title: Zusammensetzung zur Behandlung eines an Colitis ulcerosa leidenden Patienten sowie Verwendung der Zusammensetzung als Arzneimittel. Applicant: Sterna Biologicals GmbH & Co. KG. The sequence listing filed with the application follows.

SEQUENCE LISTING (1 sequence)

SEQ ID NO: 1 - DNA, 33 bp, Homo sapiens
gtggatggaggctagctacaacgagtcttggag